European Patent Application EP 4 534 663 A1, published April 9, 2025. Title: Novel variant of PTS transporter subunit EIIC and method for producing 5'-inosinic acid using the same. Applicant: DAESANG CORPORATION. The sequence listing filed with the application follows.

SEQUENCE LISTING (9 sequences)

SEQ ID NO: 1 - DNA, 2097 bp, synthetic construct
  source 1..2097: mol_type = other DNA
atggcatccgatattattagaactgacttagtcgctttagacgcagacttaggcacctcagttgaatcagtaattacccaactagccacgttagttcacgacgctggtcgcgccagcaacgtggaagaattagcgcgtcccgcaattgagcgtgaggcccaagctggcaccggagtgcctggcaaggtagcaatcccgcactgccgttccgcagcagtgagcgagccaaccttggcttttgcgcgactttctcaagcggtagatttcgcaggtcctgatggcgatgccgagttggtatttctgatcgctgccccggaaggcggcggcaaagcgcacctgaagattctttccaagcttgcgcgtgcactggtgcgccaggatttcctcgacgcgcttcgtactgcaagctcagaagaagaaatcgtcgctttagttagcgatgtcgtcagcgccgaaaagaaagcaccgaccagtgcaagctcaggtccaacagagggggcgtcgacgaacgaggcatcgacaagcgaagcatcgacaagcactgcgaaagctttgaacattgttgctgtcaccgcctgccccacaggtattgctcacacctacatggctgccgacgccctgagccaaaccgcagaaaagcgcgatgacatcaaactcacggtagaaacccaaggctcgtccaataacaccccggttgcacaatcggtcatcgacgccgctgatgccgtaatcttcgctaccgatgtgggagtacgcgaccgcgaacgcttcgctggaaaacccgtcatcgaatccggtgtaaaacgcgctatcaacgaacctgatgtcatgctgaacgaagtcgttgctgcggcgcaaaaccctaactcacacaaggttagcggtagcgcagcaatctcttctggcacggaggataccgctagccagctcagctggggcaagcgcatccagcaggccgtaatgaccggtgtgtcctacatggtgcccttcgtagccgctggcggtttgctactagcactgggctttttattcggaggcgccgatatggccaatggctggcaggccatctctacccagtattcactgaccaacctgccggggcacgaggtcgacgtcgacggtgagctcctcagctttgaacgctctggactcctgctatatatcggcgcggtgctctttgccaccggccaagcctccatgggctttatcgtctcagccctatctggctatattgcttacgctttggctgggcgccctggtatcgcgccgggctttgctggcggcgcaatcgctgtcaccgtcggcgccggcttcatcggtggtctggtcacaggtctactcgcgggtcttatcgcaatgtggatcggctcatggaaggtgccgcgctggatgaattctttaatgccagtgatgctcattccgctgttgaccactttggtggttggtctcgcaatgtacttcgtgctgggcgcaccgctggaagcgttgatgactggcctgcaaaacatgcttggtggcatgtctggttcttctgccgtggtgctgggcatcgtgctgggcctaatgatgtgttctgacctgggtggcccaattaataaggctgcctacctcttcggtaccgcagggctttccaccggtgatcaagcatccctggaaatcatggcagcgatcatggcctccggtatggttccaccaattgctttgtcgattgcaaccatcgtgcgcaagaacctctttacccctgcggagcaagaaaacggcaagtcttcctggctgatgggtctggccttcgtctccgagggcgcgattccattcgctgctgccgacccattccgcgtcattccagcgatgatggctggtggcgccactaccggtgcgctcatcatggcactcggtgtgggctcacgtgctccgcacggtggtatcttcgtgctctttgctatcgaacctatctggggctacatcgttgccatcctggtcggtactttggttgcggctgtcgccgtcatcgctttgaagcaattttggccaaataagaccatccaggaagcagcagcaaaagatgcacgagaaaaatcagccctcgcagctgcttaa

SEQ ID NO: 2 - protein, 698 aa, synthetic construct
MASDIIRTDLVALDADLGTSVESVITQLATLVHDAGRASNVEELARPAIEREAQAGTGVPGKVAIPHCRSAAVSEPTLAFARLSQAVDFAGPDGDAELVFLIAAPEGGGKAHLKILSKLARALVRQDFLDALRTASSEEEIVALVSDVVSAEKKAPTSASSGPTEGASTNEASTSEASTSTAKALNIVAVTACPTGIAHTYMAADALSQTAEKRDDIKLTVETQGSSNNTPVAQSVIDAADAVIFATDVGVRDRERFAGKPVIESGVKRAINEPDVMLNEVVAAAQNPNSHKVSGSAAISSGTEDTASQLSWGKRIQQAVMTGVSYMVPFVAAGGLLLALGFLFGGADMANGWQAISTQYSLTNLPGHEVDVDGELLSFERSGLLLYIGAVLFATGQASMGFIVSALSGYIAYALAGRPGIAPGFAGGAIAVTVGAGFIGGLVTGLLAGLIAMWIGSWKVPRWMNSLMPVMLIPLLTTLVVGLAMYFVLGAPLEALMTGLQNMLGGMSGSSAVVLGIVLGLMMCSDLGGPINKAAYLFGTAGLSTGDQASLEIMAAIMASGMVPPIALSIATIVRKNLFTPAEQENGKSSWLMGLAFVSEGAIPFAAADPFRVIPAMMAGGATTGALIMALGVGSRAPHGGIFVLFAIEPIWGYIVAILVGTLVAAVAVIALKQFWPNKTIQEAAAKDAREKSALAAA

SEQ ID NO: 3 - DNA, 2097 bp, Corynebacterium stationis
  source 1..2097: mol_type = genomic DNA
atggcatccgatattattagaactgacttagtcgctttagacgcagacttaggcacctcagttgaatcagtaattacccaactagccacgttagttcacgacgctggtcgcgccagcaacgtggaagaattagcgcgtcccgcaattgagcgtgaggcccaagctggcaccggagtgcctggcaaggtagcaatcccgcactgccgttccgcagcagtgagcgagccaaccttggcttttgcgcgactttctcaagcggtagatttcgcaggtcctgatggcgatgccgagttggtatttctgatcgctgccccggaaggcggcggcaaagcgcacctgaagattctttccaagcttgcgcgtgcactggtgcgccaggatttcctcgacgcgcttcgtactgcaagctcagaagaagaaatcgtcgctttagttagcgatgtcgtcagcgccgaaaagaaagcaccgaccagtgcaagctcaggtccaacagagggggcgtcgacgaacgaggcatcgacaagcgaagcatcgacaagcactgcgaaagctttgaacattgttgctgtcaccgcctgccccacaggtattgctcacacctacatggctgccgacgccctgagccaaaccgcagaaaagcgcgatgacatcaaactcacggtagaaacccaaggctcgtccaataacaccccggttgcacaatcggtcatcgacgccgctgatgccgtaatcttcgctaccgatgtgggagtacgcgaccgcgaacgcttcgctggaaaacccgtcatcgaatccggtgtaaaacgcgctatcaacgaacctgatgtcatgctgaacgaagccgttgctgcggcgcaaaaccctaactcacacaaggttagcggtagcgcagcaatctcttctggcacggaggataccgctagccagctcagctggggcaagcgcatccagcaggccgtaatgaccggtgtgtcctacatggtgcccttcgtagccgctggcggtttgctactagcactgggctttttattcggaggcgccgatatggccaatggctggcaggccatctctacccagtattcactgaccaacctgccggggcacgaggtcgacgtcgacggtgagctcctcagctttgaacgctctggactcctgctatatatcggcgcggtgctctttgccaccggccaagcctccatgggctttatcgtctcagccctatctggctatattgcttacgctttggctgggcgccctggtatcgcgccgggctttgctggcggcgcaatcgctgtcaccgtcggcgccggcttcatcggtggtctggtcacaggtctactcgcgggtcttatcgcaatgtggatcggctcatggaaggtgccgcgctggatgaattctttaatgccagtgatgctcattccgctgttgaccactttggtggttggtctcgcaatgtacttcgtgctgggcgcaccgctggaagcgttgatgactggcctgcaaaacatgcttggtggcatgtctggttcttctgccgtggtgctgggcatcgtgctgggcctaatgatgtgttctgacctgggtggcccaattaataaggctgcctacctcttcggtaccgcagggctttccaccggtgatcaagcatccctggaaatcatggcagcgatcatggcctccggtatggttccaccaattgctttgtcgattgcaaccatcgtgcgcaagaacctctttacccctgcggagcaagaaaacggcaagtcttcctggctgatgggtctggccttcgtctccgagggcgcgattccattcgctgctgccgacccattccgcgtcattccagcgatgatggctggtggcgccactaccggtgcgctcatcatggcactcggtgtgggctcacgtgctccgcacggtggtatcttcgtgctctttgctatcgaacctatctggggctacatcgttgccatcctggtcggtactttggttgcggctgtcgccgtcatcgctttgaagcaattttggccaaataagaccatccaggaagcagcagcaaaagatgcacgagaaaaatcagccctcgcagctgcttaa

SEQ ID NO: 4 - protein, 698 aa, Corynebacterium stationis
MASDIIRTDLVALDADLGTSVESVITQLATLVHDAGRASNVEELARPAIEREAQAGTGVPGKVAIPHCRSAAVSEPTLAFARLSQAVDFAGPDGDAELVFLIAAPEGGGKAHLKILSKLARALVRQDFLDALRTASSEEEIVALVSDVVSAEKKAPTSASSGPTEGASTNEASTSEASTSTAKALNIVAVTACPTGIAHTYMAADALSQTAEKRDDIKLTVETQGSSNNTPVAQSVIDAADAVIFATDVGVRDRERFAGKPVIESGVKRAINEPDVMLNEAVAAAQNPNSHKVSGSAAISSGTEDTASQLSWGKRIQQAVMTGVSYMVPFVAAGGLLLALGFLFGGADMANGWQAISTQYSLTNLPGHEVDVDGELLSFERSGLLLYIGAVLFATGQASMGFIVSALSGYIAYALAGRPGIAPGFAGGAIAVTVGAGFIGGLVTGLLAGLIAMWIGSWKVPRWMNSLMPVMLIPLLTTLVVGLAMYFVLGAPLEALMTGLQNMLGGMSGSSAVVLGIVLGLMMCSDLGGPINKAAYLFGTAGLSTGDQASLEIMAAIMASGMVPPIALSIATIVRKNLFTPAEQENGKSSWLMGLAFVSEGAIPFAAADPFRVIPAMMAGGATTGALIMALGVGSRAPHGGIFVLFAIEPIWGYIVAILVGTLVAAVAVIALKQFWPNKTIQEAAAKDAREKSALAAA

SEQ ID NO: 5 - DNA, 5719 bp, synthetic construct
  source 1..5719: mol_type = other DNA
tgccgcaagcactcagggcgcaagggctgctaaaggaagcggaacacgtagaaagccagtccgcagaaacggtgctgaccccggatgaatgtcagctactgggctatctggacaagggaaaacgcaagcgcaaagagaaagcaggtagcttgcagtgggcttacatggcgatagctagactgggcggttttatggacagcaagcgaaccggaattgccagctggggcgccctctggtaaggttgggaagccctgcaaagtaaactggatggctttcttgccgccaaggatctgatggcgcaggggatcaagatctgatcaagagacaggatgaggatcgtttcgcatgattgaacaagatggattgcacgcaggttctccggccgcttgggtggagaggctattcggctatgactgggcacaacagacaatcggctgctctgatgccgccgtgttccggctgtcagcgcaggggcgcccggttctttttgtcaagaccgacctgtccggtgccctgaatgaactccaagacgaggcagcgcggctatcgtggctggccacgacgggcgttccttgcgcagctgtgctcgacgttgtcactgaagcgggaagggactggctgctattgggcgaagtgccggggcaggatctcctgtcatctcaccttgctcctgccgagaaagtatccatcatggctgatgcaatgcggcggctgcatacgcttgatccggctacctgcccattcgaccaccaagcgaaacatcgcatcgagcgagcacgtactcggatggaagccggtcttgtcgatcaggatgatctggacgaagagcatcaggggctcgcgccagccgaactgttcgccaggctcaaggcgcggatgcccgacggcgaggatctcgtcgtgacccatggcgatgcctgcttgccgaatatcatggtggaaaatggccgcttttctggattcatcgactgtggccggctgggtgtggcggaccgctatcaggacatagcgttggctacccgtgatattgctgaagagcttggcggcgaatgggctgaccgcttcctcgtgctttacggtatcgccgctcccgattcgcagcgcatcgccttctatcgccttcttgacgagttcttctgagcgggactctggggttcgctagaggatcgatcctttttaacccatcacatatacctgccgttcactattatttagtgaaatgagatattatgatattttctgaattgtgattaaaaaggcaactttatgcccatgcaacagaaactataaaaaatacagagaatgaaaagaaacagatagattttttagttctttaggcccgtagtctgcaaatccttttatgattttctatcaaacaaaagaggaaaatagaccagttgcaatccaaacgagagtctaatagaatgaggtcgaaaagtaaatcgcgcgggtttgttactgataaagcaggcaagacctaaaatgtgtaaagggcaaagtgtatactttggcgtcaccccttacatattttaggtctttttttattgtgcgtaactaacttgccatcttcaaacaggagggctggaagaagcagaccgctaacacagtacataaaaaaggagacatgaacgatgaacatcaaaaagtttgcaaaacaagcaacagtattaacctttactaccgcactgctggcaggaggcgcaactcaagcgtttgcgaaagaaacgaaccaaaagccatataaggaaacatacggcatttcccatattacacgccatgatatgctgcaaatccctgaacagcaaaaaaatgaaaaatatcaagtttctgaatttgattcgtccacaattaaaaatatctcttctgcaaaaggcctggacgtttgggacagctggccattacaaaacgctgacggcactgtcgcaaactatcacggctaccacatcgtctttgcattagccggagatcctaaaaatgcggatgacacatcgatttacatgttctatcaaaaagtcggcgaaacttctattgacagctggaaaaacgctggccgcgtctttaaagacagcgacaaattcgatgcaaatgattctatcctaaaagaccaaacacaagaatggtcaggttcagccacatttacatctgacggaaaaatccgtttattctacactgatttctccggtaaacattacggcaaacaaacactgacaactgcacaagttaacgtatcagcatcagacagctctttgaacatcaacggtgtagaggattataaatcaatctttgacggtgacggaaaaacgtatcaaaatgtacagcagttcatcgatgaaggcaactacagctcaggcgacaaccatacgctgagagatcctcactacgtagaagataaaggccacaaatacttagtatttgaagcaaacactggaactgaagatggctaccaaggcgaagaatctttatttaacaaagcatactatggcaaaagcacatcattcttccgtcaagaaagtcaaaaacttctgcaaagcgataaaaaacgcacggctgagttagcaaacggcgctctcggtatgattgagctaaacgatgattacacactgaaaaaagtgatgaaaccgctgattgcatctaacacagtaacagatgaaattgaacgcgcgaacgtctttaaaatgaacggcaaatggtacctgttcactgactcccgcggatcaaaaatgacgattgacggcattacgtctaacgatatttacatgcttggttatgtttctaattctttaactggcccatacaagccgctgaacaaaactggccttgtgttaaaaatggatcttgatcctaacgatgtaacctttacttactcacacttcgctgtacctcaagcgaaaggaaacaatgtcgtgattacaagctatatgacaaacagaggattctacgcagacaaacaatcaacgtttgcgccgagcttcctgctgaacatcaaaggcaagaaaacatctgttgtcaaagacagcatccttgaacaaggacaattaacagttaacaaataaaaacgcaaaagaaaatgccgatgggtaccgagcgaaatgaccgaccaagcgacgcccaacctgccatcacgagatttcgattccaccgccgccttctatgaaaggttgggcttcggaatcgttttccgggacgccctcgcggacgtgctcatagtccacgacgcccgtgattttgtagccctggccgacggccagcaggtaggccgacaggctcatgccggccgccgccgccttttcctcaatcgctcttcgttcgtctggaaggcagtacaccttgataggtgggctgcccttcctggttggcttggtttcatcagccatccgcttgccctcatctgttacgccggcggtagccggccagcctcgcagagcaggattcccgttgagcaccgccaggtgcgaataagggacagtgaagaaggaacacccgctcgcgggtgggcctacttcacctatcctgcccggctgacgccgttggatacaccaaggaaagtctacacgaaccctttggcaaaatcctgtatatcgtgcgaaaaaggatggatataccgaaaaaatcgctataatgaccccgaagcagggttatgcagcggaaaagcgctgcttccctgctgttttgtggaatatctaccgactggaaacaggcaaatgcaggaaattactgaactgaggggacaggcgagagacgatgccaaagagctcctgaaaatctcgataactcaaaaaatacgcccggtagtgatcttatttcattatggtgaaagttggaacctcttacgtgccgatcaacgtctcattttcgccaaaagttggcccagggcttcccggtatcaacagggacaccaggatttatttattctgcgaagtgatcttccgtcacaggtatttattcggcgcaaagtgcgtcgggtgatgctgccaacttactgatttagtgtatgatggtgtttttgaggtgctccagtggcttctgtttctatcagctcctgaaaatctcgataactcaaaaaatacgcccggtagtgatcttatttcattatggtgaaagttggaacctcttacgtgccgatcaacgtctcattttcgccaaaagttggcccagggcttcccggtatcaacagggacaccaggatttatttattctgcgaagtgatcttccgtcacaggtatttattcggcgcaaagtgcgtcgggtgatgctgccaacttactgatttagtgtatgatggtgtttttgaggtgctccagtggcttctgtttctatcagggctggatgatcctccagcgcggggatctcatgctggagttcttcgcccaccccaaaaggatctaggtgaagatcctttttgataatctcatgaccaaaatcccttaacgtgagttttcgttccactgagcgtcagaccccgtagaaaagatcaaaggatcttcttgagatcctttttttctgcgcgtaatctgctgcttgcaaacaaaaaaaccaccgctaccagcggtggtttgtttgccggatcaagagctaccaactctttttccgaaggtaactggcttcagcagagcgcagataccaaatactgttcttctagtgtagccgtagttaggccaccacttcaagaactctgtagcaccgcctacatacctcgctctgctaatcctgttaccagtggctgctgccagtggcgataagtcgtgtcttaccgggttggactcaagacgatagttaccggataaggcgcagcggtcgggctgaacggggggttcgtgcacacagcccagcttggagcgaacgacctacaccgaactgagatacctacagcgtgagctatgagaaagcgccacgcttcccgaagggagaaaggcggacaggtatccggtaagcggcagggtcggaacaggagagcgcacgagggagcttccagggggaaacgcctggtatctttatagtcctgtcgggtttcgccacctctgacttgagcgtcgatttttgtgatgctcgtcaggggggcggagcctatggaaaaacgccagcaacgcggcctttttacggttcctggccttttgctggccttttgctcacatgttctttcctgcgttatcccctgattctgtggataaccgtattaccgcctttgagtgagctgataccgctcgccgcagccgaacgaccgagcgcagcgagtcagtgagcgaggaagcggaagagcgcccaatacgcaaaccgcctctccccgcgcgttggccgattcattaatgcagctggcacgacaggtttcccgactggaaagcgggcagtgagcgcaacgcaattaatgtgagttagctcactcattaggcaccccaggctttacactttatgcttccggctcgtatgttgtgtggaattgtgagcggataacaatttcacacaggaaacagctatgacatgattacgccaagcttgcatgcctgcaggtcgactctagaggatccccgggtaccgagctcgaattcactggccgtcgttttacaacgtcgtgactgggaaaaccctggcgttacccaacttaatcgccttgcagcacatccccctttcgccagctggcgtaatagcgaagaggcccgcaccgatcgcccttcccaacagttgcgcagcctgaatggcgaatggcgataagctagcttcacgc

SEQ ID NO: 6 - DNA, 20 bp, synthetic construct
  source 1..20: mol_type = other DNA
cggcaaagcgcacctgaaga

SEQ ID NO: 7 - DNA, 21 bp, synthetic construct
  source 1..21: mol_type = other DNA
ccgcagcaacgacttcgttca

SEQ ID NO: 8 - DNA, 21 bp, synthetic construct
  source 1..21: mol_type = other DNA
tgaacgaagtcgttgctgcgg

SEQ ID NO: 9 - DNA, 23 bp, synthetic construct
  source 1..23: mol_type = other DNA
tccatgagccgatccacattgcg